European Patent Application EP 4 471 146 A1, published December 4, 2024. Title: SMALL RNA DRUG FOR INHIBITING ACTIVITY OF CANCER CELLS. Applicant: Institute of Basic Medical Sciences, Chinese Academy of Medical Sciences. Application CN. The sequence listing filed with the application follows.

SEQUENCE LISTING (142 sequences)

SEQ ID NO: 1 - RNA, 18 nt, Artificial sequence
  source 1..18: mol_type = unassigned RNA
tagtggtatgattctcgc

SEQ ID NO: 2 - RNA, 21 nt, Artificial sequence
  source 1..21: mol_type = unassigned RNA
gttcagagttctacagtccga

SEQ ID NO: 3 - RNA, 20 nt, Artificial sequence
  source 1..20: mol_type = unassigned RNA
tgctgtagtaggttgtatag

SEQ ID NO: 4 - RNA, 21 nt, Artificial sequence
  source 1..21: mol_type = unassigned RNA
tgctgtagtagtttgtgctgt

SEQ ID NO: 5 - RNA, 21 nt, Artificial sequence
  source 1..21: mol_type = unassigned RNA
tcttcccagtgctctgaatgt

SEQ ID NO: 6 - RNA, 21 nt, Artificial sequence
  source 1..21: mol_type = unassigned RNA
atggttcgattccggagaggg

SEQ ID NO: 7 - RNA, 21 nt, Artificial sequence
  source 1..21: mol_type = unassigned RNA
agggttcgagtgtgagcatgc

SEQ ID NO: 8 - RNA, 20 nt, Artificial sequence
  source 1..20: mol_type = unassigned RNA
gggggcgtagctcagatggt

SEQ ID NO: 9 - RNA, 20 nt, Artificial sequence
  source 1..20: mol_type = unassigned RNA
tggaaacggctgctaatacc

SEQ ID NO: 10 - RNA, 23 nt, Artificial sequence
  source 1..23: mol_type = unassigned RNA
agctggaaacggctgctaatacc

SEQ ID NO: 11 - RNA, 21 nt, Artificial sequence
  source 1..21: mol_type = unassigned RNA
gagccccgtcgtgcccggacc

SEQ ID NO: 12 - RNA, 18 nt, Artificial sequence
  source 1..18: mol_type = unassigned RNA
acaactttcagcaacgga

SEQ ID NO: 13 - RNA, 19 nt, Artificial sequence
  source 1..19: mol_type = unassigned RNA
tacctggttgattctgcca

SEQ ID NO: 14 - RNA, 19 nt, Artificial sequence
  source 1..19: mol_type = unassigned RNA
tgtgggcactcaaagtgac

SEQ ID NO: 15 - RNA, 18 nt, Artificial sequence
  source 1..18: mol_type = unassigned RNA
tgtgggcactcaaagtga

SEQ ID NO: 16 - RNA, 24 nt, Artificial sequence
  source 1..24: mol_type = unassigned RNA
tgtgggtgcttgtgagtacggact

SEQ ID NO: 17 - RNA, 19 nt, Artificial sequence
  source 1..19: mol_type = unassigned RNA
tacctggttgatcctgcca

SEQ ID NO: 18 - RNA, 18 nt, Artificial sequence
  source 1..18: mol_type = unassigned RNA
tatctggttgattctgcc

SEQ ID NO: 19 - RNA, 31 nt, Artificial sequence
  source 1..31: mol_type = unassigned RNA
tccgttgtcgtccagcggttaggatatctgg

SEQ ID NO: 20 - RNA, 31 nt, Artificial sequence
  source 1..31: mol_type = unassigned RNA
gcgtctgtagtccaacggttaggataattgc

SEQ ID NO: 21 - RNA, 26 nt, Artificial sequence
  source 1..26: mol_type = unassigned RNA
gcgtctgtagtccaacggttaggata

SEQ ID NO: 22 - RNA, 26 nt, Artificial sequence
  source 1..26: mol_type = unassigned RNA
agggcacgtctgcctgggtgtcacgt

SEQ ID NO: 23 - RNA, 26 nt, Artificial sequence
  source 1..26: mol_type = unassigned RNA
ctgggaagtcctcgtgttgcaccctc

SEQ ID NO: 24 - RNA, 29 nt, Artificial sequence
  source 1..29: mol_type = unassigned RNA
attcggtcgggaactcaaaggagactgcc

SEQ ID NO: 25 - RNA, 29 nt, Artificial sequence
  source 1..29: mol_type = unassigned RNA
tccattgtcgtctagtccggtttaggata

SEQ ID NO: 26 - RNA, 19 nt, Artificial sequence
  source 1..19: mol_type = unassigned RNA
ggggatgtagctcagatgg

SEQ ID NO: 27 - RNA, 25 nt, Artificial sequence
  source 1..25: mol_type = unassigned RNA
gaaacgactctcggcaacggatatc

SEQ ID NO: 28 - RNA, 29 nt, Artificial sequence
  source 1..29: mol_type = unassigned RNA
cttgagttcgactctcaacgagagcacca

SEQ ID NO: 29 - RNA, 29 nt, Artificial sequence
  source 1..29: mol_type = unassigned RNA
gggattgtagttcaattggtcagagcacc

SEQ ID NO: 30 - RNA, 26 nt, Artificial sequence
  source 1..26: mol_type = unassigned RNA
tgaaacgactctcggcaacggatatc

SEQ ID NO: 31 - RNA, 29 nt, Artificial sequence
  source 1..29: mol_type = unassigned RNA
tgactctagtccgactttgtgaaatgact

SEQ ID NO: 32 - RNA, 34 nt, Artificial sequence
  source 1..34: mol_type = unassigned RNA
ggtggctgtagtttagtggtaagaattccacgtt

SEQ ID NO: 33 - RNA, 20 nt, Artificial sequence
  source 1..20: mol_type = unassigned RNA
ccgactgtttaattaaaaca

SEQ ID NO: 34 - RNA, 32 nt, Artificial sequence
  source 1..32: mol_type = unassigned RNA
tccgttgtcgtccagcggttaggatatctggc

SEQ ID NO: 35 - RNA, 28 nt, Artificial sequence
  source 1..28: mol_type = unassigned RNA
tcctctgtagttcagtcggtagaacggc

SEQ ID NO: 36 - RNA, 21 nt, Artificial sequence
  source 1..21: mol_type = unassigned RNA
tccgactgtttaattaaaaca

SEQ ID NO: 37 - RNA, 18 nt, Artificial sequence
  source 1..18: mol_type = unassigned RNA
tccgactttgtgaaatga

SEQ ID NO: 38 - RNA, 26 nt, Artificial sequence
  source 1..26: mol_type = unassigned RNA
tccgactgtttaattaaaacaaagca

SEQ ID NO: 39 - RNA, 29 nt, Artificial sequence
  source 1..29: mol_type = unassigned RNA
aggcttgtagctcaggtggttagagcgca

SEQ ID NO: 40 - RNA, 30 nt, Artificial sequence
  source 1..30: mol_type = unassigned RNA
tccgttgtcgtccagcggttaggatatctg

SEQ ID NO: 41 - RNA, 21 nt, Artificial sequence
  source 1..21: mol_type = unassigned RNA
ctctagtccgactttgtgaaa

SEQ ID NO: 42 - RNA, 19 nt, Artificial sequence
  source 1..19: mol_type = unassigned RNA
cgtcgtcgcggcgatcgtg

SEQ ID NO: 43 - RNA, 19 nt, Artificial sequence
  source 1..19: mol_type = unassigned RNA
tgaactaattcagactgtg

SEQ ID NO: 44 - RNA, 20 nt, Artificial sequence
  source 1..20: mol_type = unassigned RNA
ctctagtccgactttgtgaa

SEQ ID NO: 45 - RNA, 22 nt, Artificial sequence
  source 1..22: mol_type = unassigned RNA
caaaacgactctcggcaacgga

SEQ ID NO: 46 - RNA, 18 nt, Artificial sequence
  source 1..18: mol_type = unassigned RNA
gtaaggattgacagactg

SEQ ID NO: 47 - RNA, 19 nt, Artificial sequence
  source 1..19: mol_type = unassigned RNA
cgactctcggcaacggata

SEQ ID NO: 48 - RNA, 21 nt, Artificial sequence
  source 1..21: mol_type = unassigned RNA
gtgctctgaatgtcaaagtga

SEQ ID NO: 49 - RNA, 23 nt, Artificial sequence
  source 1..23: mol_type = unassigned RNA
aaaacgactctcggcaacggata

SEQ ID NO: 50 - RNA, 23 nt, Artificial sequence
  source 1..23: mol_type = unassigned RNA
ccctatcaactttcgatggtagg

SEQ ID NO: 51 - RNA, 20 nt, Artificial sequence
  source 1..20: mol_type = unassigned RNA
atatctcggctcacgcatcg

SEQ ID NO: 52 - RNA, 20 nt, Artificial sequence
  source 1..20: mol_type = unassigned RNA
cgttgctttttgatccttcg

SEQ ID NO: 53 - RNA, 21 nt, Artificial sequence
  source 1..21: mol_type = unassigned RNA
ctgccggcggactgctcgagc

SEQ ID NO: 54 - RNA, 18 nt, Artificial sequence
  source 1..18: mol_type = unassigned RNA
ttcacgtcgggttcacca

SEQ ID NO: 55 - RNA, 22 nt, Artificial sequence
  source 1..22: mol_type = unassigned RNA
ttgtcgtccagcggttaggata

SEQ ID NO: 56 - RNA, 27 nt, Artificial sequence
  source 1..27: mol_type = unassigned RNA
ccggagacgtcggcgggggcctcggga

SEQ ID NO: 57 - RNA, 22 nt, Artificial sequence
  source 1..22: mol_type = unassigned RNA
tgattcatgataactcgtcgga

SEQ ID NO: 58 - RNA, 19 nt, Artificial sequence
  source 1..19: mol_type = unassigned RNA
acagactgagagctctttc

SEQ ID NO: 59 - RNA, 28 nt, Artificial sequence
  source 1..28: mol_type = unassigned RNA
tccttagttcgatcctgagtgcgagctc

SEQ ID NO: 60 - RNA, 26 nt, Artificial sequence
  source 1..26: mol_type = unassigned RNA
tactgaccggggttcgtttccccgga

SEQ ID NO: 61 - RNA, 20 nt, Artificial sequence
  source 1..20: mol_type = unassigned RNA
tgataactcgtcggatcgca

SEQ ID NO: 62 - RNA, 20 nt, Artificial sequence
  source 1..20: mol_type = unassigned RNA
cccgccgcctgtttgccgac

SEQ ID NO: 63 - RNA, 19 nt, Artificial sequence
  source 1..19: mol_type = unassigned RNA
tggtccctgcggatgctca

SEQ ID NO: 64 - RNA, 23 nt, Artificial sequence
  source 1..23: mol_type = unassigned RNA
cttcactggctgtggggggaacc

SEQ ID NO: 65 - RNA, 23 nt, Artificial sequence
  source 1..23: mol_type = unassigned RNA
gtgcttgaaattgtcgggaggga

SEQ ID NO: 66 - RNA, 20 nt, Artificial sequence
  source 1..20: mol_type = unassigned RNA
atgaacaaattcagactgtg

SEQ ID NO: 67 - RNA, 20 nt, Artificial sequence
  source 1..20: mol_type = unassigned RNA
ggccgggggacggactggga

SEQ ID NO: 68 - RNA, 19 nt, Artificial sequence
  source 1..19: mol_type = unassigned RNA
acccgtcggctgtcggcga

SEQ ID NO: 69 - RNA, 19 nt, Artificial sequence
  source 1..19: mol_type = unassigned RNA
cacaccgcccgtcgctcct

SEQ ID NO: 70 - RNA, 19 nt, Artificial sequence
  source 1..19: mol_type = unassigned RNA
taatagaataggacgtgtg

SEQ ID NO: 71 - RNA, 24 nt, Artificial sequence
  source 1..24: mol_type = unassigned RNA
cagtcaactcagaactggtacgga

SEQ ID NO: 72 - RNA, 18 nt, Artificial sequence
  source 1..18: mol_type = unassigned RNA
gaaccgttgattcgcaca

SEQ ID NO: 73 - RNA, 21 nt, Artificial sequence
  source 1..21: mol_type = unassigned RNA
ccctccgaagtttccctcagg

SEQ ID NO: 74 - RNA, 19 nt, Artificial sequence
  source 1..19: mol_type = unassigned RNA
cgactctcgacaacggata

SEQ ID NO: 75 - RNA, 20 nt, Artificial sequence
  source 1..20: mol_type = unassigned RNA
ccgaccttagctcagttggt

SEQ ID NO: 76 - RNA, 19 nt, Artificial sequence
  source 1..19: mol_type = unassigned RNA
taactcgtcggatcgcacg

SEQ ID NO: 77 - RNA, 22 nt, Artificial sequence
  source 1..22: mol_type = unassigned RNA
ccggctgggggacggactggga

SEQ ID NO: 78 - RNA, 24 nt, Artificial sequence
  source 1..24: mol_type = unassigned RNA
ggtggctgtagtttagtggtgaga

SEQ ID NO: 79 - RNA, 18 nt, Artificial sequence
  source 1..18: mol_type = unassigned RNA
gtccgatcaactgtagtt

SEQ ID NO: 80 - RNA, 25 nt, Artificial sequence
  source 1..25: mol_type = unassigned RNA
ccaccgacctaagttccttggaaca

SEQ ID NO: 81 - RNA, 21 nt, Artificial sequence
  source 1..21: mol_type = unassigned RNA
tgcaaactccgaatacctaca

SEQ ID NO: 82 - RNA, 28 nt, Artificial sequence
  source 1..28: mol_type = unassigned RNA
gcgattctgacgtgcaaatcgatcgtca

SEQ ID NO: 83 - RNA, 21 nt, Artificial sequence
  source 1..21: mol_type = unassigned RNA
cgaaactcaggtgctgcaatc

SEQ ID NO: 84 - RNA, 25 nt, Artificial sequence
  source 1..25: mol_type = unassigned RNA
tcccgaacttggtggttaaactcta

SEQ ID NO: 85 - RNA, 18 nt, Artificial sequence
  source 1..18: mol_type = unassigned RNA
cttattccgtgaatcgga

SEQ ID NO: 86 - RNA, 19 nt, Artificial sequence
  source 1..19: mol_type = unassigned RNA
tcaactttcgatggtagga

SEQ ID NO: 87 - RNA, 22 nt, Artificial sequence
  source 1..22: mol_type = unassigned RNA
ttccgtccaaggctaaatactg

SEQ ID NO: 88 - RNA, 20 nt, Artificial sequence
  source 1..20: mol_type = unassigned RNA
gccggccgggggacggactg

SEQ ID NO: 89 - RNA, 21 nt, Artificial sequence
  source 1..21: mol_type = unassigned RNA
attttgttggtttctaggacc

SEQ ID NO: 90 - RNA, 23 nt, Artificial sequence
  source 1..23: mol_type = unassigned RNA
cccggtggcggacgctcttggca

SEQ ID NO: 91 - RNA, 21 nt, Artificial sequence
  source 1..21: mol_type = unassigned RNA
aaggattggctctgagggctg

SEQ ID NO: 92 - RNA, 25 nt, Artificial sequence
  source 1..25: mol_type = unassigned RNA
cgggtcgtgaacttcttttcccgga

SEQ ID NO: 93 - RNA, 18 nt, Artificial sequence
  source 1..18: mol_type = unassigned RNA
tttcggtcttattacgtt

SEQ ID NO: 94 - RNA, 20 nt, Artificial sequence
  source 1..20: mol_type = unassigned RNA
cggatatctcggctcacgca

SEQ ID NO: 95 - RNA, 19 nt, Artificial sequence
  source 1..19: mol_type = unassigned RNA
acttgagaggtgtaggata

SEQ ID NO: 96 - RNA, 20 nt, Artificial sequence
  source 1..20: mol_type = unassigned RNA
ccgaccttagctcagttggc

SEQ ID NO: 97 - RNA, 25 nt, Artificial sequence
  source 1..25: mol_type = unassigned RNA
attagtggaacgctctggaaagtgc

SEQ ID NO: 98 - RNA, 22 nt, Artificial sequence
  source 1..22: mol_type = unassigned RNA
tcgattccgggcttgcgcacca

SEQ ID NO: 99 - RNA, 22 nt, Artificial sequence
  source 1..22: mol_type = unassigned RNA
agctcgtttgattctgatttcc

SEQ ID NO: 100 - RNA, 21 nt, Artificial sequence
  source 1..21: mol_type = unassigned RNA
atccacggccataggactctg

SEQ ID NO: 101 - RNA, 21 nt, Artificial sequence
  source 1..21: mol_type = unassigned RNA
gggtgaaggacttgctccgta

SEQ ID NO: 102 - RNA, 19 nt, Artificial sequence
  source 1..19: mol_type = unassigned RNA
tgacgagtgttcttttaga

SEQ ID NO: 103 - RNA, 23 nt, Artificial sequence
  source 1..23: mol_type = unassigned RNA
tctctgaatgggggaacccactc

SEQ ID NO: 104 - RNA, 21 nt, Artificial sequence
  source 1..21: mol_type = unassigned RNA
cggactgctcgagctgcctcg

SEQ ID NO: 105 - RNA, 20 nt, Artificial sequence
  source 1..20: mol_type = unassigned RNA
cgtttggaattctggagacg

SEQ ID NO: 106 - RNA, 20 nt, Artificial sequence
  source 1..20: mol_type = unassigned RNA
ccgtcgctagcttggttgaa

SEQ ID NO: 107 - RNA, 18 nt, Artificial sequence
  source 1..18: mol_type = unassigned RNA
tccgatcaactgtagtta

SEQ ID NO: 108 - RNA, 24 nt, Artificial sequence
  source 1..24: mol_type = unassigned RNA
ctttgaatttgcttgtgtaggata

SEQ ID NO: 109 - RNA, 24 nt, Artificial sequence
  source 1..24: mol_type = unassigned RNA
gttcgattctcggcgagagagcca

SEQ ID NO: 110 - RNA, 22 nt, Artificial sequence
  source 1..22: mol_type = unassigned RNA
tcttgacgaccatagagcattg

SEQ ID NO: 111 - RNA, 20 nt, Artificial sequence
  source 1..20: mol_type = unassigned RNA
ttggtcttgtaattggaatg

SEQ ID NO: 112 - RNA, 18 nt, Artificial sequence
  source 1..18: mol_type = unassigned RNA
cgactcagaactggtacg

SEQ ID NO: 113 - RNA, 20 nt, Artificial sequence
  source 1..20: mol_type = unassigned RNA
agggaaagatgaaaaggact

SEQ ID NO: 114 - RNA, 21 nt, Artificial sequence
  source 1..21: mol_type = unassigned RNA
aaccttaacctattctcaaac

SEQ ID NO: 115 - RNA, 18 nt, Artificial sequence
  source 1..18: mol_type = unassigned RNA
tgtgtcgcttcgattcgt

SEQ ID NO: 116 - RNA, 20 nt, Artificial sequence
  source 1..20: mol_type = unassigned RNA
cgtctgcctgggtgtcacgt

SEQ ID NO: 117 - RNA, 19 nt, Artificial sequence
  source 1..19: mol_type = unassigned RNA
gtctgcctgggcgtcacgt

SEQ ID NO: 118 - RNA, 19 nt, Artificial sequence
  source 1..19: mol_type = unassigned RNA
ctggtcgggtcgtgcctcc

SEQ ID NO: 119 - RNA, 23 nt, Artificial sequence
  source 1..23: mol_type = unassigned RNA
ccccgggcgcgagcccgggcgga

SEQ ID NO: 120 - RNA, 24 nt, Artificial sequence
  source 1..24: mol_type = unassigned RNA
tctccgatcgtatagtggctagta

SEQ ID NO: 121 - RNA, 21 nt, Artificial sequence
  source 1..21: mol_type = unassigned RNA
tcccgaacccgccggctgtcg

SEQ ID NO: 122 - RNA, 24 nt, Artificial sequence
  source 1..24: mol_type = unassigned RNA
cgcgggctctgcccgttgctgcga

SEQ ID NO: 123 - RNA, 24 nt, Artificial sequence
  source 1..24: mol_type = unassigned RNA
gtttgtttgatggtatctactact

SEQ ID NO: 124 - RNA, 21 nt, Artificial sequence
  source 1..21: mol_type = unassigned RNA
cggactgctcgagctgcttcc

SEQ ID NO: 125 - RNA, 27 nt, Artificial sequence
  source 1..27: mol_type = unassigned RNA
caagtggaagtgcagtgatgtatgcag

SEQ ID NO: 126 - RNA, 19 nt, Artificial sequence
  source 1..19: mol_type = unassigned RNA
gtctttgggttccgggggg

SEQ ID NO: 127 - RNA, 21 nt, Artificial sequence
  source 1..21: mol_type = unassigned RNA
gtcccgagttcgtttctcgga

SEQ ID NO: 128 - RNA, 19 nt, Artificial sequence
  source 1..19: mol_type = unassigned RNA
ctgactcagaactggtacg

SEQ ID NO: 129 - RNA, 22 nt, Artificial sequence
  source 1..22: mol_type = unassigned RNA
catgtctgcctgggtgtcacgc

SEQ ID NO: 130 - RNA, 22 nt, Artificial sequence
  source 1..22: mol_type = unassigned RNA
tcgtgggttcgggtcccacgga

SEQ ID NO: 131 - RNA, 21 nt, Artificial sequence
  source 1..21: mol_type = unassigned RNA
tccattctcaaactttaaata

SEQ ID NO: 132 - RNA, 25 nt, Artificial sequence
  source 1..25: mol_type = unassigned RNA
ccgatgtcgtccagcggttaggata

SEQ ID NO: 133 - RNA, 19 nt, Artificial sequence
  source 1..19: mol_type = unassigned RNA
tcgcgtgccggccggggga

SEQ ID NO: 134 - RNA, 11 nt, Artificial sequence
  source 1..11: mol_type = unassigned RNA
gtctgcctggg

SEQ ID NO: 135 - RNA, 19 nt, Artificial sequence
  source 1..19: mol_type = unassigned RNA
ccgaccttagctcagttgg

SEQ ID NO: 136 - RNA, 16 nt, Artificial sequence
  source 1..16: mol_type = unassigned RNA
actcagaactggtacg

SEQ ID NO: 137 - RNA, 18 nt, Artificial sequence
  source 1..18: mol_type = unassigned RNA
tcaactttcgatggtagg

SEQ ID NO: 138 - RNA, 15 nt, Artificial sequence
  source 1..15: mol_type = unassigned RNA
tgataactcgtcgga

SEQ ID NO: 139 - RNA, 13 nt, Artificial sequence
  source 1..13: mol_type = unassigned RNA
gggggacggactg

SEQ ID NO: 140 - RNA, 13 nt, Artificial sequence
  source 1..13: mol_type = unassigned RNA
gtagctcagatgg

SEQ ID NO: 141 - RNA, 17 nt, Artificial sequence
  source 1..17: mol_type = unassigned RNA
atatctcggctcacgca

SEQ ID NO: 142 - RNA, 13 nt, Artificial sequence
  source 1..13: mol_type = unassigned RNA
aattcagactgtg